European Patent Application EP 4 613 871 A1, published September 10, 2025. Title: METHODS FOR CUT&TAG. Applicant: DIAGENODE S.A. Application EP 24162157.2, filed March 7, 2024. The sequence listing filed with the application follows.

SEQUENCE LISTING (6 sequences)

SEQ ID NO: 1 - DNA, 20 bp, Mus musculus
  source 1..20: mol_type = other DNA
gcagcatgcgttccaacaat

SEQ ID NO: 2 - DNA, 20 bp, Mus musculus
  source 1..20: mol_type = other DNA
agcgaccctagtaggaggtg

SEQ ID NO: 3 - DNA, 21 bp, Mus musculus
  source 1..21: mol_type = other DNA
gcctagtaaccgagacattga

SEQ ID NO: 4 - DNA, 20 bp, Mus musculus
  source 1..20: mol_type = other DNA
agaaagcgagattgaggaag

SEQ ID NO: 5 - DNA, 20 bp, Mus musculus
  source 1..20: mol_type = other DNA
acaaatccgagagccacaac

SEQ ID NO: 6 - DNA, 20 bp, Mus musculus
  source 1..20: mol_type = other DNA
aacaccaagagccaccaatc